European Patent Application EP 4 596 570 A1, published August 6, 2025. Title: SRC INHIBITORS AND USES THEREOF. Applicant: UNIVERSITAT DE BARCELONA. The sequence listing filed with the application follows.

SEQUENCE LISTING (2 sequences)

SEQ ID NO: 1 - protein, 30 aa, synthetic construct
MGSNKSKPKDASQRRRSLEPAENVHGAGGG

SEQ ID NO: 2 - protein, 86 aa, synthetic construct
  source 1..86: note = Src disordered region
MGSNKSKPKDASQRRRSLEPAENVHGAGGGAFPASQTPSKPASADGHRGPSAAFAPAAAEPKLFGGFNSSDTVTSPQRAGPLAGGV